European Patent Application EP 4 144 846 A1, published March 8, 2023. Title: Carbon dioxide-consuming expression system. Applicant: 350 PPM Biotech GmbH. The sequence listing filed with the application follows.

SEQUENCE LISTING (30 sequences)

SEQ ID NO: 1 - protein, 217 aa, Homo sapiens
  human growth hormone (hGH)
MATGSRTSLLLAFGLLCLPWLQEGSAFPTIPLSRLFDNAMLRAHRLHQLAFDTYQEFEEAYIPKEQKYSFLQNPQTSLCFSESIPTPSNREETQQKSNLELLRISLLLIQSWLEPVQFLRSVFANSLVYGASDSNVYDLLKDLEEGIQTLMGRLEDGSPRTGQIFKQTYSKFDTNSHNDDALLKNYGLLYCFRKDMDKVETFLRIVQCRSVEGSCGF

SEQ ID NO: 2 - protein, 231 aa, Artificial Sequence
  hGH with His-tag
MHHHHHHENLYFQSMATGSRTSLLLAFGLLCLPWLQEGSAFPTIPLSRLFDNAMLRAHRLHQLAFDTYQEFEEAYIPKEQKYSFLQNPQTSLCFSESIPTPSNREETQQKSNLELLRISLLLIQSWLEPVQFLRSVFANSLVYGASDSNVYDLLKDLEEGIQTLMGRLEDGSPRTGQIFKQTYSKFDTNSHNDDALLKNYGLLYCFRKDMDKVETFLRIVQCRSVEGSCGF

SEQ ID NO: 3 - DNA, 745 bp, Artificial Sequence
  hGH, codon-adapted for E. coli with His-Tag
gtaaaacgacggccagtgactagtatgcaccatcaccatcaccatgaaaacctttacttccagagcatggcgactgggtcccgcacttcattgttgctggcatttggacttctttgtctgccttggttgcaggaggggagtgcttttcccactataccattatctcgtctgttcgacaacgcgatgttacgggctcacagacttcaccaattagcttttgatacataccaagagtttgaggaagcctatataccaaaggaacaaaagtattcatttcttcaaaatccgcaaaccagtctttgcttcagcgagagtataccaacaccgtccaaccgtgaggaaacacaacagaagagcaacttagaacttcttcgtatttctcttttgttaatacagtcatggttggaacccgtgcagttcctgagatctgtttttgccaattcactggtctacggtgcatccgatagtaatgtgtacgatttattgaaggacttggaagagggcatccagacgttgatgggtcggcttgaagacggttcgcccagaactggccaaatatttaagcaaacatattccaagttcgacacaaattctcataatgacgatgcactgttgaagaactatggtcttttatactgtttccgcaaggatatggataaagtggaaacatttctgcgtattgtccagtgtcgctcggttgaaggttcctgcggattttagggatcccatggtcatagctgtttcc

SEQ ID NO: 4 - DNA, 20 bp, Artificial Sequence
  Primer
  misc_feature 6: /note="k = g or t"
  misc_feature 12: /note="m = a or c"
agagtktgatcmtggctcag

SEQ ID NO: 5 - DNA, 17 bp, Artificial Sequence
  Primer
  misc_feature 15: /note="r = a or g"
gacgggcggtgtgtrca

SEQ ID NO: 6 - DNA, 1402 bp, Hydrogenovibrio marinus
  16S rRNA
agagtttgatcctggctcagaatgaacgctggcggcaggcttaacacatgcaagtcgaacggtaacaggagaaagcttgctttcttgctgacgagtggcggacgggtgagtaatgtatgggaatctgccctctagttggggacaacatatggaaacgtatgctaataccgaatgtgatctacggattaaaggtgccctctccttggaaggtatcgctagaggatgagcccatattagattagctagttggtagggtaaaggcctaccaaggcgacgatctatagctggtttgagaggatgatcagccacactgggactgagacacggcccagactcctacgggaggcagcagtggggaatattgcacaatgagggaaaccttgatgcagccatgccgcgtgtgtgaagaaggcctgagggttgtaaagcactttcaattgtgaggaaagctaagtagttaatacctgcttagtgtgacgttaactttagaagaagcaccggctaactctgtgccagcagccgcggtaatacagagggtgcaagcgttattcggaattactgggcgtaaagcgcgcgtaggcggactgttaagtcggttgtgaaagccctgggctcaacctaggaattgcatccgatactggcaatctagagtttaagagagggaaggggaattccaggtgtagcagtgaaatgcgtagatatctggaggaacatcagtggcgaaggcgccttcctggcttaaaactgacgctgaggtgcgaaagcgtgggtagcgaacgggattagataccccggtagtccacgccgtaaacgatgtcaactagctgttggccttattaaaaaggttagtagcgcagctaacgcgataagttgaccgcctggggagtacggtcgcaagattaaaactcaaaggaattgacgggggcccgcacaagcggtggagcatgtggtttaattcgatgcaacgcgaagaaccttaccatcccttgacatcctgcgaactttctagagatagattggtgccttcgggaacgcagtgacaggtgctgcatggctgtcgtcagctcgtgtcgtgagatgttgggttaagtcccgcaacgagcgcaacccttatctttagttgctaccatttagttgagaactctaaagagactgccggtgataaaccggaggaaggcggggacgacgtcaagtcatcatggcccttatgggatgggctacacacgtgctacaatggggggtacaaagagcagctagctggcgacagtgcgcgaatctcataaaacccttcgtagtccggattggagtctgcaactcgactccatgaagtcggaatcgctagtaatcgtgaatcagaatgtcacggtgaatacgttcccgggccttgtacacaccgcccgtc

SEQ ID NO: 7 - DNA, 886 bp, Artificial Sequence
  GFP expression cassette
tctagataatgaattctataggtaccttgacagctagctcagtcctaggtataatgctagcactagagaaagaggagaaatactagtatgtggagccacccgcagttcgaaaaaggatcaagcaaaggagaagaacttttcactggagttgtcccaattcttgttgaattagatggtgatgttaatgggcacaaattttctgtccgtggagagggtgaaggtgatgctacaaacggaaaacttacccttaaatttatttgcactactggaaaactacctgttccatggccaacacttgtcactactctcacttatggtgttcaatgcttttcccgttatccggatcatatgaaacggcatgactttttcaagagtgccatgcccgaaggttatgtacaggaacgcactatatctttcaaagatgacgggacttacaagacgcgtgctgaagtcaagtttgaaggtgatacccttgttaatcgtatcgagttaaaaggtattgattttaaagaagatggaaacattctcggacacaaacttgagtacaactttaactcacacaatgtatacatcacggcagacaaacaaaagaatggaatcaaagctaacttcaaaattcgccacaacgttgaagatggttccgttcaactagcagaccattatcaacaaaatactccaattggcgatggccctgtccttttaccagacaaccattacctgtctacacaatctgtcctttcgaaagatcccaacgaaaagcgtgaccacatggtccttcttgagtttgtaactgctgctgggattacacatggcatggatgagctctacaaataaggatcctgaagatccaacgctcggttgccgccgggcgttttttattctgcag

SEQ ID NO: 8 - DNA, 35 bp, Artificial Sequence
  Promoter J23119
ttgacagctagctcagtcctaggtataatgctagc

SEQ ID NO: 9 - DNA, 35 bp, Artificial Sequence
  Promoter J23111
ttgacggctagctcagtcctaggtatagtgctagc

SEQ ID NO: 10 - DNA, 35 bp, Artificial Sequence
  Promoter J23114
tttatggctagctcagtcctaggtacaatgctagc

SEQ ID NO: 11 - DNA, 28 bp, Artificial Sequence
  RBS BBa_B0034
tctagagaaagaggagaaatactagatg

SEQ ID NO: 12 - DNA, 28 bp, Artificial Sequence
  RBS BBa_B0064
tctagagaaagaggggaaatactagatg

SEQ ID NO: 13 - DNA, 30 bp, Artificial Sequence
  RBS BBa_B0031
tctagagtcacacaggaaacctactagatg

SEQ ID NO: 14 - DNA, 44 bp, Artificial Sequence
  RBS_ribDG
actagagacggtaaataacaaaagaggggagggacactagtatg

SEQ ID NO: 15 - DNA, 57 bp, Artificial Sequence
  Primer DNA_039
cttgacggctagctcagtcctaggtatagtgctagcactagagaaagaggggaaata

SEQ ID NO: 16 - DNA, 65 bp, Artificial Sequence
  Primer DNA_040
ctagtatttcccctctttctctagtgctagcactatacctaggactgagctagccgtcaaggtac

SEQ ID NO: 17 - DNA, 58 bp, Artificial Sequence
  Primer DNA_041
ctttatggctagctcagtcctaggtacaatgctagcactagagtcacacaggaaacca

SEQ ID NO: 18 - DNA, 66 bp, Artificial Sequence
  Primer DNA_042
ctagtggtttcctgtgtgactctagtgctagcattgtacctaggactgagctagccataaaggtac

SEQ ID NO: 19 - DNA, 72 bp, Artificial Sequence
  Primer DNA_043
cttgacagctagctcagtcctaggtataatgctagcactagagacggtaaataacaaaagaggggagggaca

SEQ ID NO: 20 - DNA, 37 bp, Artificial Sequence
  Primer DNA_051
tttggtctcactagtacgttgtgtctcaaaatctctg

SEQ ID NO: 21 - DNA, 37 bp, Artificial Sequence
  Primer DNA_052
tttggtctcaagcttccagatgtatgctcttctgctc

SEQ ID NO: 22 - DNA, 8410 bp, Artificial Sequence
  plasmid pHM38
agtcctcgtctcgccctcgaattagcccgcttaatgagcgggctttttttgaattaattctcgcgagctggcacgacaggtttcccgactggaaagcgggcagtgagcgcaacgcaattaatgtaagttagcgcgaattgcaagctggccgacgcgctgggctacgtcttgctggcgttcgggagcagaagagcatacatctggaagcaaagccaggaaagcggcctatggagctgtgcggcagcgctcagtaggcaatttttcaaaatattgttaagccttttctgagcatggtatttttcatggtattaccaattagcaggaaaataagccattgaatataaaagataaaaatgtcttgtttacaatagagtggggggggtcagcctgccgccttgggccgggtgatgtcgtacttgcccgccgcgaactcggttaccgtccagcccagcgcgaccagctccggcaacgcctcgcgcacccgctggcggcgcttgcgcatggtcgaaccactggcctctgacggccagacatagccgcacaaggtatctatggaagccttgccggttttgccggggtcgatccagccacacagccgctggtgcagcaggcgggcggtttcgctgtccagcgcccgcacctcgtccatgctgatgcgcacatgctggccgccacccatgacggcctgcgcgatcaaggggttcagggccacgtacaggcgcccgtccgcctcgtcgctggcgtactccgacagcagccgaaacccctgccgcttgcggccattctgggcgatgatggataccttccaaaggcgctcgatgcagtcctgtatgtgcttgagcgccccaccactatcgacctctgccccgatttcctttgccagcgcccgatagctacctttgaccaccatggcatcagcggtgacggcctcccacttgggttccaggaacagccggagctgccgtccgccttcggtcttgggttccgggccaagcactaggccattaggcccagccatggccaccagcccttgcaggatgcgcagatcatcagcgcccagcggctccgggccgctgaactcgatccgcttgccgtcgccgtagtcatacgtcacgtccagcttgctgcgcttgcgctcgccccgcttgagggcacggaacaggccgggggccagacagtgcgccgggtcgtgtcggacgtggctgaggctgtgcttgttcttaggcttcaccacggggcacccccttgctcttgcgctgcctctccagcacggcgggcttgagcaccccgccgtcatgccgcctgaaccaccgatcagcgaacggtgcgccatagttggccttgctcacaccgaagcggacgaagaaccggcgctggtcgtcgtccacaccccattcctcggcctcggcgctggtcatgctcgacaggtaggactgccagcggatgttatcgaccagtaccgagctgccccggctggcctgctgctggtcgcctgcgcccatcatggccgcgcccttgctggcatggtgcaggaacacgatagagcacccggtatcggcggcgatggcctccatgcgaccgatgacctgggccatggggccgctggcgttttcttcctcgatgtggaaccggcgcagcgtgtccagcaccatcaggcggcggccctcggcggcgcgcttgaggccgtcgaaccactccggggccatgatgttgggcaggctgccgatcagcggctggatcagcaggccgtcagccacggcttgccgttcctcggcgctgaggtgcgccccaagggcgtgcaggcggtgatgaatggcggtgggcgggtcttcggcgggcaggtagatcaccgggccggtgggcagttcgcccacctccagcagatccggcccgcctgcaatctgtgcggccagttgcagggccagcatggatttaccggcaccaccgggcgacaccagcgccccgaccgtaccggccaccatgttgggcaaaacgtagtccagcggtggcggcgctgctgcgaacgcctccagaatattgataggcttatgggtagccattgattgcctcctttgcaggcagttggtggttaggcgctggcggggtcactacccccgccctgcgccgctctgagttcttccaggcactcgcgcagcgcctcgtattcgtcgtcggtcagccagaacttgcgctgacgcatccctttggccttcatgcgctcggcatatcgcgcttggcgtacagcgtcagggctggccagcaggtcgccggtctgcttgtccttttggtctttcatatcagtcaccgagaaacttgccggggccgaaaggcttgtcttcgcggaacaaggacaaggtgcagccgtcaaggttaaggctggccatatcagcgactgaaaagcggccagcctcggccttgtttgacgtataaccaaagccaccgggcaaccaatagcccttgtcacttttgatcaggtagaccgaccctgaagcgcttttttcgtattccataaaacccccttctgtgcgtgagtactcatagtataacaggcgtgagtaccaacgcaagcactacatgctgaaatctggcccgcccctgtccatgcctcgctggcggggtgccggtgcccgtgccagctcggcccgcgcaagctggacgctgggcagacccatgaccttgctgacggtgcgctcgatgtaatccgcttcgtggccgggcttgcgctctgccagcgctgggctggcctcggccatggccttgccgatttcctcggcactgcggccccggctggccagcttctgcgcggcgataaagtcgcacttgctgaggtcatcaccgaagcgcttgaccagcccggccatctcgctgcggtactcgtccagcgccgtgcgccggtggcggctaagctgccgctcggacagttcgaggctggccagcctgcgggccttctcctgctgccgctgggcctgctcgatctgctggccagcctgctgcaccagcgccgggccagcggtggcggtcttgcccttggattcacgcagcagcacccacggctgataaccggcgcgggtggtgtgcttgtccttgcggttggtgaagcccgccaagcggccatagtggcggctgtcggcgctggccgggtcggcgtcgtactcgctggccagcgtccgggcaatctgcccccgaagttcaccgcctgcggcgtcggccaccttgacccatgcctgatagttcttcgggctggtttccactaccagggcaggctcccggccctcggctttcatgtcatccaggtcaaactcgctgaggtcgtccaccagcaccagaccatgccgctcctgctcggcgggcctgatatacacgtcattgccctgggcattcatccgcttgagccatggcgtgttctggagcacttcggcggctgaccattcccggttcatcatctggccggtggtggcgtccctgacgccgatatcgaagcgctcacagcccatggccttgagctgtcggcctatggcctgcaaagtcctgtcgttcttcatcgggccaccaagcgcagccagatcgagccgtcctcggttgtcagtggcgtcaggtcgagcaagagcaacgatgcgatcagcagcaccaccgtaggcatcatggaagccagcatcacggttagccatagcttccagtgccacccccgcgacgcgctccgggcgctctgcgcggcgctgctcacctcggcggctacctcccgcaactctttggccagctccacccatgccgcccctgtctggcgctgggctttcagccactccgccgcctgcgcctcgctggcctgctgggtctggctcatgacctgccgggcttcgtcggccagtgtcgccatgctctgggccagcggttcgatctgctccgctaactcgttgatgcctctggatttcttcactctgtcgattgcgttcatggtctattgcctcccggtattcctgtaagtcgatgatctgggcgttggcggtgtcgatgttcagggccacgtctgcccggtcggtgcggatgccccggccttccatctccaccacgttcggccccaggtgaacaccgggcaggcgctcgatgccctgcgcctcaagtgttctgtggtcaatgcgggcgtcgtggcctgcccgctctaatgcccggttggcatggtcggcccatgcctcgcgggtctgctcaagccatgccttgggcttgagcgcttcggtcttctgtgccccgcccttctccggggtcttgccgttgtaccgcttgaaccactgagcggcgggccgctcgatgccgtcattgatccgctcggagatcatcaggtggcagtgcgggttctcgccgccaccggcatggatggccagcgtatacggcaggcgctcggcaccggtcaggtgctgggcgaactcggacgccagcgccttctgctggtcgagggtcagctcgaccggcagggcaaattcgacctccttgaacagccgcccattggcgcgttcatacaggtcggcagcatcccagtagtcggcgggccgctcgacgaactccggcatgtgcccggattcggcgtgcaagacttcatccatgtcgcgggcatacttgccttcgcgctggatgaagtcggccttggccctggccgattggccgcccgacctgctgccggttttcgccgtaaggtgataaatcgccatgctgcctcgctgttgcttttgcttttcggctccatgcaatggccctcggagagcgcaccgcccgaagggtggccgttaggccagtttctcgaagagaaaccggtaagtgcgccctcccctacaaagtagggtcgggattgccgccgctgtgcctccatgatagcctacgagacagcacattaacaatggggtgtcaagatggttaaggggagcaacaaggcggcggatcggctggccaagctcgaagaacaacgagcgcgaatcaatgccgaaattcagcgggtgcgggcaagggaacagcagcaagagcgcaagaacgaaacaaggcgcaaggtgctggtgggggccatgattttggccaaggtgaacagcagcgagtggccggaggatcggctcatggcggcaatggatgcgtaccttgaacgcgaccacgaccgcgccttgttcggtctgccgccacgccagaaggatgagccgggctgaatgatcgaccgagacaggccctgcggggctgcacacgcgcccccacccttcgggtagggggaaaggccgctaaagcggctaaaagcgctccagcgtatttctgcggggtttggtgtggggtttagcgggctttgcccgcctttccccctgccgcgcagcggtggggcggtgtgtagcctagcgcagcgaatagaccagctatccggcctctggccgggcatattgggcaagggcagcagcgccccacaagggcgctgataaccgcgcctagtggattattcttagataatcatggatggatttttccaacaccccgccagcccccgcccctgctgggtttgcaggtttgggggcgtgacagttattgcaggggttcgtgacagttattgcaggggggcgtgacagttattgcaggggttcgtgacagttagtacgggagtgacgggcactggctggcaatgtctagcaacggcaggcatttcggctgagggtaaaagaactttccgctaagcgatagactgtatgtaaacacagtattgcaaggacgcggaacatgcctcatgtggcggccctcgcgagaattaattcagataaaaaaaatccttagctttcgctaaggatgatttctagcgatgaccctgctgattggttcgctgaccgtagactggttggcttggtttcatcagccatccgcttgccctcatctgttacgccggcggtagccggccagcctcgcagagcaggattcccgttgagcaccgccaggtgcgaataagggacagtgaagaaggaacacccgctcgcgggtgggcctacttcacctatcctgcccggctgacgccgttggatacaccaaggaaagtctacacgaaccctttggcaaaatcctgtatatcgtgcgacatcgcgcgcgcgcgcgcggatgctagtacgttgtgtctcaaaatctctgatgttacattgcacaagataaaaatatatcatcatgaacaataaaactgtctgcttacataaacagtaatacaaggggtgttatgagccatattcaacgggaaacgtcttgctcgaggccgcgattaaattccaacatggatgctgatttatatgggtataaatgggctcgcgataatgtcgggcaatcaggtgcgacaatctatcgattgtatgggaagcccgatgcgccagagttgtttctgaaacatggcaaaggtagcgttgccaatgatgttacagatgagatggtcagactaaactggctgacggaatttatgcctcttccgaccatcaagcattttatccgtactcctgatgatgcatggttactcaccactgcgatccccgggaaaacagcattccaggtattagaagaatatcctgattcaggtgaaaatattgttgatgcgctggcagtgttcctgcgccggttgcattcgattcctgtttgtaattgtccttttaacagcgatcgcgtatttcgtctcgctcaggcgcaatcacgaatgaataacggtttggttgatgcgagtgattttgatgacgagcgtaatggctggcctgttgaacaagtctggaaagaaatgcataagcttttgccattctcaccggattcagtcgtcactcatggtgatttctcacttgataaccttatttttgacgaggggaaattaataggttgtattgatgttggacgagtcggaatcgcagaccgataccaggatcttgccatcctatggaactgcctcggtgagttttctccttcattacagaaacggctttttcaaaaatatggtattgataatcctgatatgaataaattgcagtttcatttgatgctcgatgagtttttctaatcagaattggttaattggttgtaacactggcagagcattacgctgacttgacgggacggcggctttgttgaataaatcgaacttttgctgagttgaaggatcagatcacgcatcttcccgacaacgcagaccgttccgtggcaaagcaaaagttcaaaatcaccaactggtccacctacaacaaagctctcatcaaccgtggctccctcactttctggctggatgatggggcgattcaggcctggtatgagtcagcaacaccttcttcacgaggcagacctcagcgctattctgaccttgccatcacgactgtgctggtcattaaacgcgtattcaggctgaccctgcgcgctgcgcagggctttattgattccatttttacactgatgaatgttccgttgcgctgcccggattacagatcctctagataatgaattctataggtaccttgacagctagctcagtcctaggtataatgctagcactagagaaagaggagaaatactagtatgtggagccacccgcagttcgaaaaaggatcaagcaaaggagaagaacttttcactggagttgtcccaattcttgttgaattagatggtgatgttaatgggcacaaattttctgtccgtggagagggtgaaggtgatgctacaaacggaaaacttacccttaaatttatttgcactactggaaaactacctgttccatggccaacacttgtcactactctcacttatggtgttcaatgcttttcccgttatccggatcatatgaaacggcatgactttttcaagagtgccatgcccgaaggttatgtacaggaacgcactatatctttcaaagatgacgggacttacaagacgcgtgctgaagtcaagtttgaaggtgatacccttgttaatcgtatcgagttaaaaggtattgattttaaagaagatggaaacattctcggacacaaacttgagtacaactttaactcacacaatgtatacatcacggcagacaaacaaaagaatggaatcaaagctaacttcaaaattcgccacaacgttgaagatggttccgttcaactagcagaccattatcaacaaaatactccaattggcgatggccctgtccttttaccagacaaccattacctgtctacacaatctgtcctttcgaaagatcccaacgaaaagcgtgaccacatggtccttcttgagtttgtaactgctgctgggattacacatggcatggatgagctctacaaataaggatcctgaagatccaacgctcggttgccgccgggcgttttttattctgcaggagcagaagagcatacatctggaagctttctagaatcgggggcccccggggggattctagaacaatgga

SEQ ID NO: 23 - DNA, 8410 bp, Artificial Sequence
  plasmid pHM39
agtcctcgtctcgccctcgaattagcccgcttaatgagcgggctttttttgaattaattctcgcgagctggcacgacaggtttcccgactggaaagcgggcagtgagcgcaacgcaattaatgtaagttagcgcgaattgcaagctggccgacgcgctgggctacgtcttgctggcgttcgggagcagaagagcatacatctggaagcaaagccaggaaagcggcctatggagctgtgcggcagcgctcagtaggcaatttttcaaaatattgttaagccttttctgagcatggtatttttcatggtattaccaattagcaggaaaataagccattgaatataaaagataaaaatgtcttgtttacaatagagtggggggggtcagcctgccgccttgggccgggtgatgtcgtacttgcccgccgcgaactcggttaccgtccagcccagcgcgaccagctccggcaacgcctcgcgcacccgctggcggcgcttgcgcatggtcgaaccactggcctctgacggccagacatagccgcacaaggtatctatggaagccttgccggttttgccggggtcgatccagccacacagccgctggtgcagcaggcgggcggtttcgctgtccagcgcccgcacctcgtccatgctgatgcgcacatgctggccgccacccatgacggcctgcgcgatcaaggggttcagggccacgtacaggcgcccgtccgcctcgtcgctggcgtactccgacagcagccgaaacccctgccgcttgcggccattctgggcgatgatggataccttccaaaggcgctcgatgcagtcctgtatgtgcttgagcgccccaccactatcgacctctgccccgatttcctttgccagcgcccgatagctacctttgaccaccatggcatcagcggtgacggcctcccacttgggttccaggaacagccggagctgccgtccgccttcggtcttgggttccgggccaagcactaggccattaggcccagccatggccaccagcccttgcaggatgcgcagatcatcagcgcccagcggctccgggccgctgaactcgatccgcttgccgtcgccgtagtcatacgtcacgtccagcttgctgcgcttgcgctcgccccgcttgagggcacggaacaggccgggggccagacagtgcgccgggtcgtgtcggacgtggctgaggctgtgcttgttcttaggcttcaccacggggcacccccttgctcttgcgctgcctctccagcacggcgggcttgagcaccccgccgtcatgccgcctgaaccaccgatcagcgaacggtgcgccatagttggccttgctcacaccgaagcggacgaagaaccggcgctggtcgtcgtccacaccccattcctcggcctcggcgctggtcatgctcgacaggtaggactgccagcggatgttatcgaccagtaccgagctgccccggctggcctgctgctggtcgcctgcgcccatcatggccgcgcccttgctggcatggtgcaggaacacgatagagcacccggtatcggcggcgatggcctccatgcgaccgatgacctgggccatggggccgctggcgttttcttcctcgatgtggaaccggcgcagcgtgtccagcaccatcaggcggcggccctcggcggcgcgcttgaggccgtcgaaccactccggggccatgatgttgggcaggctgccgatcagcggctggatcagcaggccgtcagccacggcttgccgttcctcggcgctgaggtgcgccccaagggcgtgcaggcggtgatgaatggcggtgggcgggtcttcggcgggcaggtagatcaccgggccggtgggcagttcgcccacctccagcagatccggcccgcctgcaatctgtgcggccagttgcagggccagcatggatttaccggcaccaccgggcgacaccagcgccccgaccgtaccggccaccatgttgggcaaaacgtagtccagcggtggcggcgctgctgcgaacgcctccagaatattgataggcttatgggtagccattgattgcctcctttgcaggcagttggtggttaggcgctggcggggtcactacccccgccctgcgccgctctgagttcttccaggcactcgcgcagcgcctcgtattcgtcgtcggtcagccagaacttgcgctgacgcatccctttggccttcatgcgctcggcatatcgcgcttggcgtacagcgtcagggctggccagcaggtcgccggtctgcttgtccttttggtctttcatatcagtcaccgagaaacttgccggggccgaaaggcttgtcttcgcggaacaaggacaaggtgcagccgtcaaggttaaggctggccatatcagcgactgaaaagcggccagcctcggccttgtttgacgtataaccaaagccaccgggcaaccaatagcccttgtcacttttgatcaggtagaccgaccctgaagcgcttttttcgtattccataaaacccccttctgtgcgtgagtactcatagtataacaggcgtgagtaccaacgcaagcactacatgctgaaatctggcccgcccctgtccatgcctcgctggcggggtgccggtgcccgtgccagctcggcccgcgcaagctggacgctgggcagacccatgaccttgctgacggtgcgctcgatgtaatccgcttcgtggccgggcttgcgctctgccagcgctgggctggcctcggccatggccttgccgatttcctcggcactgcggccccggctggccagcttctgcgcggcgataaagtcgcacttgctgaggtcatcaccgaagcgcttgaccagcccggccatctcgctgcggtactcgtccagcgccgtgcgccggtggcggctaagctgccgctcggacagttcgaggctggccagcctgcgggccttctcctgctgccgctgggcctgctcgatctgctggccagcctgctgcaccagcgccgggccagcggtggcggtcttgcccttggattcacgcagcagcacccacggctgataaccggcgcgggtggtgtgcttgtccttgcggttggtgaagcccgccaagcggccatagtggcggctgtcggcgctggccgggtcggcgtcgtactcgctggccagcgtccgggcaatctgcccccgaagttcaccgcctgcggcgtcggccaccttgacccatgcctgatagttcttcgggctggtttccactaccagggcaggctcccggccctcggctttcatgtcatccaggtcaaactcgctgaggtcgtccaccagcaccagaccatgccgctcctgctcggcgggcctgatatacacgtcattgccctgggcattcatccgcttgagccatggcgtgttctggagcacttcggcggctgaccattcccggttcatcatctggccggtggtggcgtccctgacgccgatatcgaagcgctcacagcccatggccttgagctgtcggcctatggcctgcaaagtcctgtcgttcttcatcgggccaccaagcgcagccagatcgagccgtcctcggttgtcagtggcgtcaggtcgagcaagagcaacgatgcgatcagcagcaccaccgtaggcatcatggaagccagcatcacggttagccatagcttccagtgccacccccgcgacgcgctccgggcgctctgcgcggcgctgctcacctcggcggctacctcccgcaactctttggccagctccacccatgccgcccctgtctggcgctgggctttcagccactccgccgcctgcgcctcgctggcctgctgggtctggctcatgacctgccgggcttcgtcggccagtgtcgccatgctctgggccagcggttcgatctgctccgctaactcgttgatgcctctggatttcttcactctgtcgattgcgttcatggtctattgcctcccggtattcctgtaagtcgatgatctgggcgttggcggtgtcgatgttcagggccacgtctgcccggtcggtgcggatgccccggccttccatctccaccacgttcggccccaggtgaacaccgggcaggcgctcgatgccctgcgcctcaagtgttctgtggtcaatgcgggcgtcgtggcctgcccgctctaatgcccggttggcatggtcggcccatgcctcgcgggtctgctcaagccatgccttgggcttgagcgcttcggtcttctgtgccccgcccttctccggggtcttgccgttgtaccgcttgaaccactgagcggcgggccgctcgatgccgtcattgatccgctcggagatcatcaggtggcagtgcgggttctcgccgccaccggcatggatggccagcgtatacggcaggcgctcggcaccggtcaggtgctgggcgaactcggacgccagcgccttctgctggtcgagggtcagctcgaccggcagggcaaattcgacctccttgaacagccgcccattggcgcgttcatacaggtcggcagcatcccagtagtcggcgggccgctcgacgaactccggcatgtgcccggattcggcgtgcaagacttcatccatgtcgcgggcatacttgccttcgcgctggatgaagtcggccttggccctggccgattggccgcccgacctgctgccggttttcgccgtaaggtgataaatcgccatgctgcctcgctgttgcttttgcttttcggctccatgcaatggccctcggagagcgcaccgcccgaagggtggccgttaggccagtttctcgaagagaaaccggtaagtgcgccctcccctacaaagtagggtcgggattgccgccgctgtgcctccatgatagcctacgagacagcacattaacaatggggtgtcaagatggttaaggggagcaacaaggcggcggatcggctggccaagctcgaagaacaacgagcgcgaatcaatgccgaaattcagcgggtgcgggcaagggaacagcagcaagagcgcaagaacgaaacaaggcgcaaggtgctggtgggggccatgattttggccaaggtgaacagcagcgagtggccggaggatcggctcatggcggcaatggatgcgtaccttgaacgcgaccacgaccgcgccttgttcggtctgccgccacgccagaaggatgagccgggctgaatgatcgaccgagacaggccctgcggggctgcacacgcgcccccacccttcgggtagggggaaaggccgctaaagcggctaaaagcgctccagcgtatttctgcggggtttggtgtggggtttagcgggctttgcccgcctttccccctgccgcgcagcggtggggcggtgtgtagcctagcgcagcgaatagaccagctatccggcctctggccgggcatattgggcaagggcagcagcgccccacaagggcgctgataaccgcgcctagtggattattcttagataatcatggatggatttttccaacaccccgccagcccccgcccctgctgggtttgcaggtttgggggcgtgacagttattgcaggggttcgtgacagttattgcaggggggcgtgacagttattgcaggggttcgtgacagttagtacgggagtgacgggcactggctggcaatgtctagcaacggcaggcatttcggctgagggtaaaagaactttccgctaagcgatagactgtatgtaaacacagtattgcaaggacgcggaacatgcctcatgtggcggccctcgcgagaattaattcagataaaaaaaatccttagctttcgctaaggatgatttctagcgatgaccctgctgattggttcgctgaccgtagactggttggcttggtttcatcagccatccgcttgccctcatctgttacgccggcggtagccggccagcctcgcagagcaggattcccgttgagcaccgccaggtgcgaataagggacagtgaagaaggaacacccgctcgcgggtgggcctacttcacctatcctgcccggctgacgccgttggatacaccaaggaaagtctacacgaaccctttggcaaaatcctgtatatcgtgcgacatcgcgcgcgcgcgcgcggatgctagtacgttgtgtctcaaaatctctgatgttacattgcacaagataaaaatatatcatcatgaacaataaaactgtctgcttacataaacagtaatacaaggggtgttatgagccatattcaacgggaaacgtcttgctcgaggccgcgattaaattccaacatggatgctgatttatatgggtataaatgggctcgcgataatgtcgggcaatcaggtgcgacaatctatcgattgtatgggaagcccgatgcgccagagttgtttctgaaacatggcaaaggtagcgttgccaatgatgttacagatgagatggtcagactaaactggctgacggaatttatgcctcttccgaccatcaagcattttatccgtactcctgatgatgcatggttactcaccactgcgatccccgggaaaacagcattccaggtattagaagaatatcctgattcaggtgaaaatattgttgatgcgctggcagtgttcctgcgccggttgcattcgattcctgtttgtaattgtccttttaacagcgatcgcgtatttcgtctcgctcaggcgcaatcacgaatgaataacggtttggttgatgcgagtgattttgatgacgagcgtaatggctggcctgttgaacaagtctggaaagaaatgcataagcttttgccattctcaccggattcagtcgtcactcatggtgatttctcacttgataaccttatttttgacgaggggaaattaataggttgtattgatgttggacgagtcggaatcgcagaccgataccaggatcttgccatcctatggaactgcctcggtgagttttctccttcattacagaaacggctttttcaaaaatatggtattgataatcctgatatgaataaattgcagtttcatttgatgctcgatgagtttttctaatcagaattggttaattggttgtaacactggcagagcattacgctgacttgacgggacggcggctttgttgaataaatcgaacttttgctgagttgaaggatcagatcacgcatcttcccgacaacgcagaccgttccgtggcaaagcaaaagttcaaaatcaccaactggtccacctacaacaaagctctcatcaaccgtggctccctcactttctggctggatgatggggcgattcaggcctggtatgagtcagcaacaccttcttcacgaggcagacctcagcgctattctgaccttgccatcacgactgtgctggtcattaaacgcgtattcaggctgaccctgcgcgctgcgcagggctttattgattccatttttacactgatgaatgttccgttgcgctgcccggattacagatcctctagataatgaattctataggtaccttgacggctagctcagtcctaggtatagtgctagcactagagaaagaggggaaatactagtatgtggagccacccgcagttcgaaaaaggatcaagcaaaggagaagaacttttcactggagttgtcccaattcttgttgaattagatggtgatgttaatgggcacaaattttctgtccgtggagagggtgaaggtgatgctacaaacggaaaacttacccttaaatttatttgcactactggaaaactacctgttccatggccaacacttgtcactactctcacttatggtgttcaatgcttttcccgttatccggatcatatgaaacggcatgactttttcaagagtgccatgcccgaaggttatgtacaggaacgcactatatctttcaaagatgacgggacttacaagacgcgtgctgaagtcaagtttgaaggtgatacccttgttaatcgtatcgagttaaaaggtattgattttaaagaagatggaaacattctcggacacaaacttgagtacaactttaactcacacaatgtatacatcacggcagacaaacaaaagaatggaatcaaagctaacttcaaaattcgccacaacgttgaagatggttccgttcaactagcagaccattatcaacaaaatactccaattggcgatggccctgtccttttaccagacaaccattacctgtctacacaatctgtcctttcgaaagatcccaacgaaaagcgtgaccacatggtccttcttgagtttgtaactgctgctgggattacacatggcatggatgagctctacaaataaggatcctgaagatccaacgctcggttgccgccgggcgttttttattctgcaggagcagaagagcatacatctggaagctttctagaatcgggggcccccggggggattctagaacaatgga

SEQ ID NO: 24 - DNA, 8411 bp, Artificial Sequence
  plasmid pHM40
agtcctcgtctcgccctcgaattagcccgcttaatgagcgggctttttttgaattaattctcgcgagctggcacgacaggtttcccgactggaaagcgggcagtgagcgcaacgcaattaatgtaagttagcgcgaattgcaagctggccgacgcgctgggctacgtcttgctggcgttcgggagcagaagagcatacatctggaagcaaagccaggaaagcggcctatggagctgtgcggcagcgctcagtaggcaatttttcaaaatattgttaagccttttctgagcatggtatttttcatggtattaccaattagcaggaaaataagccattgaatataaaagataaaaatgtcttgtttacaatagagtggggggggtcagcctgccgccttgggccgggtgatgtcgtacttgcccgccgcgaactcggttaccgtccagcccagcgcgaccagctccggcaacgcctcgcgcacccgctggcggcgcttgcgcatggtcgaaccactggcctctgacggccagacatagccgcacaaggtatctatggaagccttgccggttttgccggggtcgatccagccacacagccgctggtgcagcaggcgggcggtttcgctgtccagcgcccgcacctcgtccatgctgatgcgcacatgctggccgccacccatgacggcctgcgcgatcaaggggttcagggccacgtacaggcgcccgtccgcctcgtcgctggcgtactccgacagcagccgaaacccctgccgcttgcggccattctgggcgatgatggataccttccaaaggcgctcgatgcagtcctgtatgtgcttgagcgccccaccactatcgacctctgccccgatttcctttgccagcgcccgatagctacctttgaccaccatggcatcagcggtgacggcctcccacttgggttccaggaacagccggagctgccgtccgccttcggtcttgggttccgggccaagcactaggccattaggcccagccatggccaccagcccttgcaggatgcgcagatcatcagcgcccagcggctccgggccgctgaactcgatccgcttgccgtcgccgtagtcatacgtcacgtccagcttgctgcgcttgcgctcgccccgcttgagggcacggaacaggccgggggccagacagtgcgccgggtcgtgtcggacgtggctgaggctgtgcttgttcttaggcttcaccacggggcacccccttgctcttgcgctgcctctccagcacggcgggcttgagcaccccgccgtcatgccgcctgaaccaccgatcagcgaacggtgcgccatagttggccttgctcacaccgaagcggacgaagaaccggcgctggtcgtcgtccacaccccattcctcggcctcggcgctggtcatgctcgacaggtaggactgccagcggatgttatcgaccagtaccgagctgccccggctggcctgctgctggtcgcctgcgcccatcatggccgcgcccttgctggcatggtgcaggaacacgatagagcacccggtatcggcggcgatggcctccatgcgaccgatgacctgggccatggggccgctggcgttttcttcctcgatgtggaaccggcgcagcgtgtccagcaccatcaggcggcggccctcggcggcgcgcttgaggccgtcgaaccactccggggccatgatgttgggcaggctgccgatcagcggctggatcagcaggccgtcagccacggcttgccgttcctcggcgctgaggtgcgccccaagggcgtgcaggcggtgatgaatggcggtgggcgggtcttcggcgggcaggtagatcaccgggccggtgggcagttcgcccacctccagcagatccggcccgcctgcaatctgtgcggccagttgcagggccagcatggatttaccggcaccaccgggcgacaccagcgccccgaccgtaccggccaccatgttgggcaaaacgtagtccagcggtggcggcgctgctgcgaacgcctccagaatattgataggcttatgggtagccattgattgcctcctttgcaggcagttggtggttaggcgctggcggggtcactacccccgccctgcgccgctctgagttcttccaggcactcgcgcagcgcctcgtattcgtcgtcggtcagccagaacttgcgctgacgcatccctttggccttcatgcgctcggcatatcgcgcttggcgtacagcgtcagggctggccagcaggtcgccggtctgcttgtccttttggtctttcatatcagtcaccgagaaacttgccggggccgaaaggcttgtcttcgcggaacaaggacaaggtgcagccgtcaaggttaaggctggccatatcagcgactgaaaagcggccagcctcggccttgtttgacgtataaccaaagccaccgggcaaccaatagcccttgtcacttttgatcaggtagaccgaccctgaagcgcttttttcgtattccataaaacccccttctgtgcgtgagtactcatagtataacaggcgtgagtaccaacgcaagcactacatgctgaaatctggcccgcccctgtccatgcctcgctggcggggtgccggtgcccgtgccagctcggcccgcgcaagctggacgctgggcagacccatgaccttgctgacggtgcgctcgatgtaatccgcttcgtggccgggcttgcgctctgccagcgctgggctggcctcggccatggccttgccgatttcctcggcactgcggccccggctggccagcttctgcgcggcgataaagtcgcacttgctgaggtcatcaccgaagcgcttgaccagcccggccatctcgctgcggtactcgtccagcgccgtgcgccggtggcggctaagctgccgctcggacagttcgaggctggccagcctgcgggccttctcctgctgccgctgggcctgctcgatctgctggccagcctgctgcaccagcgccgggccagcggtggcggtcttgcccttggattcacgcagcagcacccacggctgataaccggcgcgggtggtgtgcttgtccttgcggttggtgaagcccgccaagcggccatagtggcggctgtcggcgctggccgggtcggcgtcgtactcgctggccagcgtccgggcaatctgcccccgaagttcaccgcctgcggcgtcggccaccttgacccatgcctgatagttcttcgggctggtttccactaccagggcaggctcccggccctcggctttcatgtcatccaggtcaaactcgctgaggtcgtccaccagcaccagaccatgccgctcctgctcggcgggcctgatatacacgtcattgccctgggcattcatccgcttgagccatggcgtgttctggagcacttcggcggctgaccattcccggttcatcatctggccggtggtggcgtccctgacgccgatatcgaagcgctcacagcccatggccttgagctgtcggcctatggcctgcaaagtcctgtcgttcttcatcgggccaccaagcgcagccagatcgagccgtcctcggttgtcagtggcgtcaggtcgagcaagagcaacgatgcgatcagcagcaccaccgtaggcatcatggaagccagcatcacggttagccatagcttccagtgccacccccgcgacgcgctccgggcgctctgcgcggcgctgctcacctcggcggctacctcccgcaactctttggccagctccacccatgccgcccctgtctggcgctgggctttcagccactccgccgcctgcgcctcgctggcctgctgggtctggctcatgacctgccgggcttcgtcggccagtgtcgccatgctctgggccagcggttcgatctgctccgctaactcgttgatgcctctggatttcttcactctgtcgattgcgttcatggtctattgcctcccggtattcctgtaagtcgatgatctgggcgttggcggtgtcgatgttcagggccacgtctgcccggtcggtgcggatgccccggccttccatctccaccacgttcggccccaggtgaacaccgggcaggcgctcgatgccctgcgcctcaagtgttctgtggtcaatgcgggcgtcgtggcctgcccgctctaatgcccggttggcatggtcggcccatgcctcgcgggtctgctcaagccatgccttgggcttgagcgcttcggtcttctgtgccccgcccttctccggggtcttgccgttgtaccgcttgaaccactgagcggcgggccgctcgatgccgtcattgatccgctcggagatcatcaggtggcagtgcgggttctcgccgccaccggcatggatggccagcgtatacggcaggcgctcggcaccggtcaggtgctgggcgaactcggacgccagcgccttctgctggtcgagggtcagctcgaccggcagggcaaattcgacctccttgaacagccgcccattggcgcgttcatacaggtcggcagcatcccagtagtcggcgggccgctcgacgaactccggcatgtgcccggattcggcgtgcaagacttcatccatgtcgcgggcatacttgccttcgcgctggatgaagtcggccttggccctggccgattggccgcccgacctgctgccggttttcgccgtaaggtgataaatcgccatgctgcctcgctgttgcttttgcttttcggctccatgcaatggccctcggagagcgcaccgcccgaagggtggccgttaggccagtttctcgaagagaaaccggtaagtgcgccctcccctacaaagtagggtcgggattgccgccgctgtgcctccatgatagcctacgagacagcacattaacaatggggtgtcaagatggttaaggggagcaacaaggcggcggatcggctggccaagctcgaagaacaacgagcgcgaatcaatgccgaaattcagcgggtgcgggcaagggaacagcagcaagagcgcaagaacgaaacaaggcgcaaggtgctggtgggggccatgattttggccaaggtgaacagcagcgagtggccggaggatcggctcatggcggcaatggatgcgtaccttgaacgcgaccacgaccgcgccttgttcggtctgccgccacgccagaaggatgagccgggctgaatgatcgaccgagacaggccctgcggggctgcacacgcgcccccacccttcgggtagggggaaaggccgctaaagcggctaaaagcgctccagcgtatttctgcggggtttggtgtggggtttagcgggctttgcccgcctttccccctgccgcgcagcggtggggcggtgtgtagcctagcgcagcgaatagaccagctatccggcctctggccgggcatattgggcaagggcagcagcgccccacaagggcgctgataaccgcgcctagtggattattcttagataatcatggatggatttttccaacaccccgccagcccccgcccctgctgggtttgcaggtttgggggcgtgacagttattgcaggggttcgtgacagttattgcaggggggcgtgacagttattgcaggggttcgtgacagttagtacgggagtgacgggcactggctggcaatgtctagcaacggcaggcatttcggctgagggtaaaagaactttccgctaagcgatagactgtatgtaaacacagtattgcaaggacgcggaacatgcctcatgtggcggccctcgcgagaattaattcagataaaaaaaatccttagctttcgctaaggatgatttctagcgatgaccctgctgattggttcgctgaccgtagactggttggcttggtttcatcagccatccgcttgccctcatctgttacgccggcggtagccggccagcctcgcagagcaggattcccgttgagcaccgccaggtgcgaataagggacagtgaagaaggaacacccgctcgcgggtgggcctacttcacctatcctgcccggctgacgccgttggatacaccaaggaaagtctacacgaaccctttggcaaaatcctgtatatcgtgcgacatcgcgcgcgcgcgcgcggatgctagtacgttgtgtctcaaaatctctgatgttacattgcacaagataaaaatatatcatcatgaacaataaaactgtctgcttacataaacagtaatacaaggggtgttatgagccatattcaacgggaaacgtcttgctcgaggccgcgattaaattccaacatggatgctgatttatatgggtataaatgggctcgcgataatgtcgggcaatcaggtgcgacaatctatcgattgtatgggaagcccgatgcgccagagttgtttctgaaacatggcaaaggtagcgttgccaatgatgttacagatgagatggtcagactaaactggctgacggaatttatgcctcttccgaccatcaagcattttatccgtactcctgatgatgcatggttactcaccactgcgatccccgggaaaacagcattccaggtattagaagaatatcctgattcaggtgaaaatattgttgatgcgctggcagtgttcctgcgccggttgcattcgattcctgtttgtaattgtccttttaacagcgatcgcgtatttcgtctcgctcaggcgcaatcacgaatgaataacggtttggttgatgcgagtgattttgatgacgagcgtaatggctggcctgttgaacaagtctggaaagaaatgcataagcttttgccattctcaccggattcagtcgtcactcatggtgatttctcacttgataaccttatttttgacgaggggaaattaataggttgtattgatgttggacgagtcggaatcgcagaccgataccaggatcttgccatcctatggaactgcctcggtgagttttctccttcattacagaaacggctttttcaaaaatatggtattgataatcctgatatgaataaattgcagtttcatttgatgctcgatgagtttttctaatcagaattggttaattggttgtaacactggcagagcattacgctgacttgacgggacggcggctttgttgaataaatcgaacttttgctgagttgaaggatcagatcacgcatcttcccgacaacgcagaccgttccgtggcaaagcaaaagttcaaaatcaccaactggtccacctacaacaaagctctcatcaaccgtggctccctcactttctggctggatgatggggcgattcaggcctggtatgagtcagcaacaccttcttcacgaggcagacctcagcgctattctgaccttgccatcacgactgtgctggtcattaaacgcgtattcaggctgaccctgcgcgctgcgcagggctttattgattccatttttacactgatgaatgttccgttgcgctgcccggattacagatcctctagataatgaattctataggtacctttatggctagctcagtcctaggtacaatgctagcactagagtcacacaggaaaccactagtatgtggagccacccgcagttcgaaaaaggatcaagcaaaggagaagaacttttcactggagttgtcccaattcttgttgaattagatggtgatgttaatgggcacaaattttctgtccgtggagagggtgaaggtgatgctacaaacggaaaacttacccttaaatttatttgcactactggaaaactacctgttccatggccaacacttgtcactactctcacttatggtgttcaatgcttttcccgttatccggatcatatgaaacggcatgactttttcaagagtgccatgcccgaaggttatgtacaggaacgcactatatctttcaaagatgacgggacttacaagacgcgtgctgaagtcaagtttgaaggtgatacccttgttaatcgtatcgagttaaaaggtattgattttaaagaagatggaaacattctcggacacaaacttgagtacaactttaactcacacaatgtatacatcacggcagacaaacaaaagaatggaatcaaagctaacttcaaaattcgccacaacgttgaagatggttccgttcaactagcagaccattatcaacaaaatactccaattggcgatggccctgtccttttaccagacaaccattacctgtctacacaatctgtcctttcgaaagatcccaacgaaaagcgtgaccacatggtccttcttgagtttgtaactgctgctgggattacacatggcatggatgagctctacaaataaggatcctgaagatccaacgctcggttgccgccgggcgttttttattctgcaggagcagaagagcatacatctggaagctttctagaatcgggggcccccggggggattctagaacaatgga

SEQ ID NO: 25 - DNA, 8425 bp, Artificial Sequence
  plasmid pHM41
agtcctcgtctcgccctcgaattagcccgcttaatgagcgggctttttttgaattaattctcgcgagctggcacgacaggtttcccgactggaaagcgggcagtgagcgcaacgcaattaatgtaagttagcgcgaattgcaagctggccgacgcgctgggctacgtcttgctggcgttcgggagcagaagagcatacatctggaagcaaagccaggaaagcggcctatggagctgtgcggcagcgctcagtaggcaatttttcaaaatattgttaagccttttctgagcatggtatttttcatggtattaccaattagcaggaaaataagccattgaatataaaagataaaaatgtcttgtttacaatagagtggggggggtcagcctgccgccttgggccgggtgatgtcgtacttgcccgccgcgaactcggttaccgtccagcccagcgcgaccagctccggcaacgcctcgcgcacccgctggcggcgcttgcgcatggtcgaaccactggcctctgacggccagacatagccgcacaaggtatctatggaagccttgccggttttgccggggtcgatccagccacacagccgctggtgcagcaggcgggcggtttcgctgtccagcgcccgcacctcgtccatgctgatgcgcacatgctggccgccacccatgacggcctgcgcgatcaaggggttcagggccacgtacaggcgcccgtccgcctcgtcgctggcgtactccgacagcagccgaaacccctgccgcttgcggccattctgggcgatgatggataccttccaaaggcgctcgatgcagtcctgtatgtgcttgagcgccccaccactatcgacctctgccccgatttcctttgccagcgcccgatagctacctttgaccaccatggcatcagcggtgacggcctcccacttgggttccaggaacagccggagctgccgtccgccttcggtcttgggttccgggccaagcactaggccattaggcccagccatggccaccagcccttgcaggatgcgcagatcatcagcgcccagcggctccgggccgctgaactcgatccgcttgccgtcgccgtagtcatacgtcacgtccagcttgctgcgcttgcgctcgccccgcttgagggcacggaacaggccgggggccagacagtgcgccgggtcgtgtcggacgtggctgaggctgtgcttgttcttaggcttcaccacggggcacccccttgctcttgcgctgcctctccagcacggcgggcttgagcaccccgccgtcatgccgcctgaaccaccgatcagcgaacggtgcgccatagttggccttgctcacaccgaagcggacgaagaaccggcgctggtcgtcgtccacaccccattcctcggcctcggcgctggtcatgctcgacaggtaggactgccagcggatgttatcgaccagtaccgagctgccccggctggcctgctgctggtcgcctgcgcccatcatggccgcgcccttgctggcatggtgcaggaacacgatagagcacccggtatcggcggcgatggcctccatgcgaccgatgacctgggccatggggccgctggcgttttcttcctcgatgtggaaccggcgcagcgtgtccagcaccatcaggcggcggccctcggcggcgcgcttgaggccgtcgaaccactccggggccatgatgttgggcaggctgccgatcagcggctggatcagcaggccgtcagccacggcttgccgttcctcggcgctgaggtgcgccccaagggcgtgcaggcggtgatgaatggcggtgggcgggtcttcggcgggcaggtagatcaccgggccggtgggcagttcgcccacctccagcagatccggcccgcctgcaatctgtgcggccagttgcagggccagcatggatttaccggcaccaccgggcgacaccagcgccccgaccgtaccggccaccatgttgggcaaaacgtagtccagcggtggcggcgctgctgcgaacgcctccagaatattgataggcttatgggtagccattgattgcctcctttgcaggcagttggtggttaggcgctggcggggtcactacccccgccctgcgccgctctgagttcttccaggcactcgcgcagcgcctcgtattcgtcgtcggtcagccagaacttgcgctgacgcatccctttggccttcatgcgctcggcatatcgcgcttggcgtacagcgtcagggctggccagcaggtcgccggtctgcttgtccttttggtctttcatatcagtcaccgagaaacttgccggggccgaaaggcttgtcttcgcggaacaaggacaaggtgcagccgtcaaggttaaggctggccatatcagcgactgaaaagcggccagcctcggccttgtttgacgtataaccaaagccaccgggcaaccaatagcccttgtcacttttgatcaggtagaccgaccctgaagcgcttttttcgtattccataaaacccccttctgtgcgtgagtactcatagtataacaggcgtgagtaccaacgcaagcactacatgctgaaatctggcccgcccctgtccatgcctcgctggcggggtgccggtgcccgtgccagctcggcccgcgcaagctggacgctgggcagacccatgaccttgctgacggtgcgctcgatgtaatccgcttcgtggccgggcttgcgctctgccagcgctgggctggcctcggccatggccttgccgatttcctcggcactgcggccccggctggccagcttctgcgcggcgataaagtcgcacttgctgaggtcatcaccgaagcgcttgaccagcccggccatctcgctgcggtactcgtccagcgccgtgcgccggtggcggctaagctgccgctcggacagttcgaggctggccagcctgcgggccttctcctgctgccgctgggcctgctcgatctgctggccagcctgctgcaccagcgccgggccagcggtggcggtcttgcccttggattcacgcagcagcacccacggctgataaccggcgcgggtggtgtgcttgtccttgcggttggtgaagcccgccaagcggccatagtggcggctgtcggcgctggccgggtcggcgtcgtactcgctggccagcgtccgggcaatctgcccccgaagttcaccgcctgcggcgtcggccaccttgacccatgcctgatagttcttcgggctggtttccactaccagggcaggctcccggccctcggctttcatgtcatccaggtcaaactcgctgaggtcgtccaccagcaccagaccatgccgctcctgctcggcgggcctgatatacacgtcattgccctgggcattcatccgcttgagccatggcgtgttctggagcacttcggcggctgaccattcccggttcatcatctggccggtggtggcgtccctgacgccgatatcgaagcgctcacagcccatggccttgagctgtcggcctatggcctgcaaagtcctgtcgttcttcatcgggccaccaagcgcagccagatcgagccgtcctcggttgtcagtggcgtcaggtcgagcaagagcaacgatgcgatcagcagcaccaccgtaggcatcatggaagccagcatcacggttagccatagcttccagtgccacccccgcgacgcgctccgggcgctctgcgcggcgctgctcacctcggcggctacctcccgcaactctttggccagctccacccatgccgcccctgtctggcgctgggctttcagccactccgccgcctgcgcctcgctggcctgctgggtctggctcatgacctgccgggcttcgtcggccagtgtcgccatgctctgggccagcggttcgatctgctccgctaactcgttgatgcctctggatttcttcactctgtcgattgcgttcatggtctattgcctcccggtattcctgtaagtcgatgatctgggcgttggcggtgtcgatgttcagggccacgtctgcccggtcggtgcggatgccccggccttccatctccaccacgttcggccccaggtgaacaccgggcaggcgctcgatgccctgcgcctcaagtgttctgtggtcaatgcgggcgtcgtggcctgcccgctctaatgcccggttggcatggtcggcccatgcctcgcgggtctgctcaagccatgccttgggcttgagcgcttcggtcttctgtgccccgcccttctccggggtcttgccgttgtaccgcttgaaccactgagcggcgggccgctcgatgccgtcattgatccgctcggagatcatcaggtggcagtgcgggttctcgccgccaccggcatggatggccagcgtatacggcaggcgctcggcaccggtcaggtgctgggcgaactcggacgccagcgccttctgctggtcgagggtcagctcgaccggcagggcaaattcgacctccttgaacagccgcccattggcgcgttcatacaggtcggcagcatcccagtagtcggcgggccgctcgacgaactccggcatgtgcccggattcggcgtgcaagacttcatccatgtcgcgggcatacttgccttcgcgctggatgaagtcggccttggccctggccgattggccgcccgacctgctgccggttttcgccgtaaggtgataaatcgccatgctgcctcgctgttgcttttgcttttcggctccatgcaatggccctcggagagcgcaccgcccgaagggtggccgttaggccagtttctcgaagagaaaccggtaagtgcgccctcccctacaaagtagggtcgggattgccgccgctgtgcctccatgatagcctacgagacagcacattaacaatggggtgtcaagatggttaaggggagcaacaaggcggcggatcggctggccaagctcgaagaacaacgagcgcgaatcaatgccgaaattcagcgggtgcgggcaagggaacagcagcaagagcgcaagaacgaaacaaggcgcaaggtgctggtgggggccatgattttggccaaggtgaacagcagcgagtggccggaggatcggctcatggcggcaatggatgcgtaccttgaacgcgaccacgaccgcgccttgttcggtctgccgccacgccagaaggatgagccgggctgaatgatcgaccgagacaggccctgcggggctgcacacgcgcccccacccttcgggtagggggaaaggccgctaaagcggctaaaagcgctccagcgtatttctgcggggtttggtgtggggtttagcgggctttgcccgcctttccccctgccgcgcagcggtggggcggtgtgtagcctagcgcagcgaatagaccagctatccggcctctggccgggcatattgggcaagggcagcagcgccccacaagggcgctgataaccgcgcctagtggattattcttagataatcatggatggatttttccaacaccccgccagcccccgcccctgctgggtttgcaggtttgggggcgtgacagttattgcaggggttcgtgacagttattgcaggggggcgtgacagttattgcaggggttcgtgacagttagtacgggagtgacgggcactggctggcaatgtctagcaacggcaggcatttcggctgagggtaaaagaactttccgctaagcgatagactgtatgtaaacacagtattgcaaggacgcggaacatgcctcatgtggcggccctcgcgagaattaattcagataaaaaaaatccttagctttcgctaaggatgatttctagcgatgaccctgctgattggttcgctgaccgtagactggttggcttggtttcatcagccatccgcttgccctcatctgttacgccggcggtagccggccagcctcgcagagcaggattcccgttgagcaccgccaggtgcgaataagggacagtgaagaaggaacacccgctcgcgggtgggcctacttcacctatcctgcccggctgacgccgttggatacaccaaggaaagtctacacgaaccctttggcaaaatcctgtatatcgtgcgacatcgcgcgcgcgcgcgcggatgctagtacgttgtgtctcaaaatctctgatgttacattgcacaagataaaaatatatcatcatgaacaataaaactgtctgcttacataaacagtaatacaaggggtgttatgagccatattcaacgggaaacgtcttgctcgaggccgcgattaaattccaacatggatgctgatttatatgggtataaatgggctcgcgataatgtcgggcaatcaggtgcgacaatctatcgattgtatgggaagcccgatgcgccagagttgtttctgaaacatggcaaaggtagcgttgccaatgatgttacagatgagatggtcagactaaactggctgacggaatttatgcctcttccgaccatcaagcattttatccgtactcctgatgatgcatggttactcaccactgcgatccccgggaaaacagcattccaggtattagaagaatatcctgattcaggtgaaaatattgttgatgcgctggcagtgttcctgcgccggttgcattcgattcctgtttgtaattgtccttttaacagcgatcgcgtatttcgtctcgctcaggcgcaatcacgaatgaataacggtttggttgatgcgagtgattttgatgacgagcgtaatggctggcctgttgaacaagtctggaaagaaatgcataagcttttgccattctcaccggattcagtcgtcactcatggtgatttctcacttgataaccttatttttgacgaggggaaattaataggttgtattgatgttggacgagtcggaatcgcagaccgataccaggatcttgccatcctatggaactgcctcggtgagttttctccttcattacagaaacggctttttcaaaaatatggtattgataatcctgatatgaataaattgcagtttcatttgatgctcgatgagtttttctaatcagaattggttaattggttgtaacactggcagagcattacgctgacttgacgggacggcggctttgttgaataaatcgaacttttgctgagttgaaggatcagatcacgcatcttcccgacaacgcagaccgttccgtggcaaagcaaaagttcaaaatcaccaactggtccacctacaacaaagctctcatcaaccgtggctccctcactttctggctggatgatggggcgattcaggcctggtatgagtcagcaacaccttcttcacgaggcagacctcagcgctattctgaccttgccatcacgactgtgctggtcattaaacgcgtattcaggctgaccctgcgcgctgcgcagggctttattgattccatttttacactgatgaatgttccgttgcgctgcccggattacagatcctctagataatgaattctataggtaccttgacagctagctcagtcctaggtataatgctagcactagagacggtaaataacaaaagaggggagggacactagtatgtggagccacccgcagttcgaaaaaggatcaagcaaaggagaagaacttttcactggagttgtcccaattcttgttgaattagatggtgatgttaatgggcacaaattttctgtccgtggagagggtgaaggtgatgctacaaacggaaaacttacccttaaatttatttgcactactggaaaactacctgttccatggccaacacttgtcactactctcacttatggtgttcaatgcttttcccgttatccggatcatatgaaacggcatgactttttcaagagtgccatgcccgaaggttatgtacaggaacgcactatatctttcaaagatgacgggacttacaagacgcgtgctgaagtcaagtttgaaggtgatacccttgttaatcgtatcgagttaaaaggtattgattttaaagaagatggaaacattctcggacacaaacttgagtacaactttaactcacacaatgtatacatcacggcagacaaacaaaagaatggaatcaaagctaacttcaaaattcgccacaacgttgaagatggttccgttcaactagcagaccattatcaacaaaatactccaattggcgatggccctgtccttttaccagacaaccattacctgtctacacaatctgtcctttcgaaagatcccaacgaaaagcgtgaccacatggtccttcttgagtttgtaactgctgctgggattacacatggcatggatgagctctacaaataaggatcctgaagatccaacgctcggttgccgccgggcgttttttattctgcaggagcagaagagcatacatctggaagctttctagaatcgggggcccccggggggattctagaacaatgga

SEQ ID NO: 26 - DNA, 7632 bp, Artificial Sequence
  plasmid pHM42
agtcctcgtctcgccctcgaattagcccgcttaatgagcgggctttttttgaattaattctcgcgagctggcacgacaggtttcccgactggaaagcgggcagtgagcgcaacgcaattaatgtaagttagcgcgaattgcaagctggccgacgcgctgggctacgtcttgctggcgttcgggagcagaagagcatacatctggaagcaaagccaggaaagcggcctatggagctgtgcggcagcgctcagtaggcaatttttcaaaatattgttaagccttttctgagcatggtatttttcatggtattaccaattagcaggaaaataagccattgaatataaaagataaaaatgtcttgtttacaatagagtggggggggtcagcctgccgccttgggccgggtgatgtcgtacttgcccgccgcgaactcggttaccgtccagcccagcgcgaccagctccggcaacgcctcgcgcacccgctggcggcgcttgcgcatggtcgaaccactggcctctgacggccagacatagccgcacaaggtatctatggaagccttgccggttttgccggggtcgatccagccacacagccgctggtgcagcaggcgggcggtttcgctgtccagcgcccgcacctcgtccatgctgatgcgcacatgctggccgccacccatgacggcctgcgcgatcaaggggttcagggccacgtacaggcgcccgtccgcctcgtcgctggcgtactccgacagcagccgaaacccctgccgcttgcggccattctgggcgatgatggataccttccaaaggcgctcgatgcagtcctgtatgtgcttgagcgccccaccactatcgacctctgccccgatttcctttgccagcgcccgatagctacctttgaccaccatggcatcagcggtgacggcctcccacttgggttccaggaacagccggagctgccgtccgccttcggtcttgggttccgggccaagcactaggccattaggcccagccatggccaccagcccttgcaggatgcgcagatcatcagcgcccagcggctccgggccgctgaactcgatccgcttgccgtcgccgtagtcatacgtcacgtccagcttgctgcgcttgcgctcgccccgcttgagggcacggaacaggccgggggccagacagtgcgccgggtcgtgtcggacgtggctgaggctgtgcttgttcttaggcttcaccacggggcacccccttgctcttgcgctgcctctccagcacggcgggcttgagcaccccgccgtcatgccgcctgaaccaccgatcagcgaacggtgcgccatagttggccttgctcacaccgaagcggacgaagaaccggcgctggtcgtcgtccacaccccattcctcggcctcggcgctggtcatgctcgacaggtaggactgccagcggatgttatcgaccagtaccgagctgccccggctggcctgctgctggtcgcctgcgcccatcatggccgcgcccttgctggcatggtgcaggaacacgatagagcacccggtatcggcggcgatggcctccatgcgaccgatgacctgggccatggggccgctggcgttttcttcctcgatgtggaaccggcgcagcgtgtccagcaccatcaggcggcggccctcggcggcgcgcttgaggccgtcgaaccactccggggccatgatgttgggcaggctgccgatcagcggctggatcagcaggccgtcagccacggcttgccgttcctcggcgctgaggtgcgccccaagggcgtgcaggcggtgatgaatggcggtgggcgggtcttcggcgggcaggtagatcaccgggccggtgggcagttcgcccacctccagcagatccggcccgcctgcaatctgtgcggccagttgcagggccagcatggatttaccggcaccaccgggcgacaccagcgccccgaccgtaccggccaccatgttgggcaaaacgtagtccagcggtggcggcgctgctgcgaacgcctccagaatattgataggcttatgggtagccattgattgcctcctttgcaggcagttggtggttaggcgctggcggggtcactacccccgccctgcgccgctctgagttcttccaggcactcgcgcagcgcctcgtattcgtcgtcggtcagccagaacttgcgctgacgcatccctttggccttcatgcgctcggcatatcgcgcttggcgtacagcgtcagggctggccagcaggtcgccggtctgcttgtccttttggtctttcatatcagtcaccgagaaacttgccggggccgaaaggcttgtcttcgcggaacaaggacaaggtgcagccgtcaaggttaaggctggccatatcagcgactgaaaagcggccagcctcggccttgtttgacgtataaccaaagccaccgggcaaccaatagcccttgtcacttttgatcaggtagaccgaccctgaagcgcttttttcgtattccataaaacccccttctgtgcgtgagtactcatagtataacaggcgtgagtaccaacgcaagcactacatgctgaaatctggcccgcccctgtccatgcctcgctggcggggtgccggtgcccgtgccagctcggcccgcgcaagctggacgctgggcagacccatgaccttgctgacggtgcgctcgatgtaatccgcttcgtggccgggcttgcgctctgccagcgctgggctggcctcggccatggccttgccgatttcctcggcactgcggccccggctggccagcttctgcgcggcgataaagtcgcacttgctgaggtcatcaccgaagcgcttgaccagcccggccatctcgctgcggtactcgtccagcgccgtgcgccggtggcggctaagctgccgctcggacagttcgaggctggccagcctgcgggccttctcctgctgccgctgggcctgctcgatctgctggccagcctgctgcaccagcgccgggccagcggtggcggtcttgcccttggattcacgcagcagcacccacggctgataaccggcgcgggtggtgtgcttgtccttgcggttggtgaagcccgccaagcggccatagtggcggctgtcggcgctggccgggtcggcgtcgtactcgctggccagcgtccgggcaatctgcccccgaagttcaccgcctgcggcgtcggccaccttgacccatgcctgatagttcttcgggctggtttccactaccagggcaggctcccggccctcggctttcatgtcatccaggtcaaactcgctgaggtcgtccaccagcaccagaccatgccgctcctgctcggcgggcctgatatacacgtcattgccctgggcattcatccgcttgagccatggcgtgttctggagcacttcggcggctgaccattcccggttcatcatctggccggtggtggcgtccctgacgccgatatcgaagcgctcacagcccatggccttgagctgtcggcctatggcctgcaaagtcctgtcgttcttcatcgggccaccaagcgcagccagatcgagccgtcctcggttgtcagtggcgtcaggtcgagcaagagcaacgatgcgatcagcagcaccaccgtaggcatcatggaagccagcatcacggttagccatagcttccagtgccacccccgcgacgcgctccgggcgctctgcgcggcgctgctcacctcggcggctacctcccgcaactctttggccagctccacccatgccgcccctgtctggcgctgggctttcagccactccgccgcctgcgcctcgctggcctgctgggtctggctcatgacctgccgggcttcgtcggccagtgtcgccatgctctgggccagcggttcgatctgctccgctaactcgttgatgcctctggatttcttcactctgtcgattgcgttcatggtctattgcctcccggtattcctgtaagtcgatgatctgggcgttggcggtgtcgatgttcagggccacgtctgcccggtcggtgcggatgccccggccttccatctccaccacgttcggccccaggtgaacaccgggcaggcgctcgatgccctgcgcctcaagtgttctgtggtcaatgcgggcgtcgtggcctgcccgctctaatgcccggttggcatggtcggcccatgcctcgcgggtctgctcaagccatgccttgggcttgagcgcttcggtcttctgtgccccgcccttctccggggtcttgccgttgtaccgcttgaaccactgagcggcgggccgctcgatgccgtcattgatccgctcggagatcatcaggtggcagtgcgggttctcgccgccaccggcatggatggccagcgtatacggcaggcgctcggcaccggtcaggtgctgggcgaactcggacgccagcgccttctgctggtcgagggtcagctcgaccggcagggcaaattcgacctccttgaacagccgcccattggcgcgttcatacaggtcggcagcatcccagtagtcggcgggccgctcgacgaactccggcatgtgcccggattcggcgtgcaagacttcatccatgtcgcgggcatacttgccttcgcgctggatgaagtcggccttggccctggccgattggccgcccgacctgctgccggttttcgccgtaaggtgataaatcgccatgctgcctcgctgttgcttttgcttttcggctccatgcaatggccctcggagagcgcaccgcccgaagggtggccgttaggccagtttctcgaagagaaaccggtaagtgcgccctcccctacaaagtagggtcgggattgccgccgctgtgcctccatgatagcctacgagacagcacattaacaatggggtgtcaagatggttaaggggagcaacaaggcggcggatcggctggccaagctcgaagaacaacgagcgcgaatcaatgccgaaattcagcgggtgcgggcaagggaacagcagcaagagcgcaagaacgaaacaaggcgcaaggtgctggtgggggccatgattttggccaaggtgaacagcagcgagtggccggaggatcggctcatggcggcaatggatgcgtaccttgaacgcgaccacgaccgcgccttgttcggtctgccgccacgccagaaggatgagccgggctgaatgatcgaccgagacaggccctgcggggctgcacacgcgcccccacccttcgggtagggggaaaggccgctaaagcggctaaaagcgctccagcgtatttctgcggggtttggtgtggggtttagcgggctttgcccgcctttccccctgccgcgcagcggtggggcggtgtgtagcctagcgcagcgaatagaccagctatccggcctctggccgggcatattgggcaagggcagcagcgccccacaagggcgctgataaccgcgcctagtggattattcttagataatcatggatggatttttccaacaccccgccagcccccgcccctgctgggtttgcaggtttgggggcgtgacagttattgcaggggttcgtgacagttattgcaggggggcgtgacagttattgcaggggttcgtgacagttagtacgggagtgacgggcactggctggcaatgtctagcaacggcaggcatttcggctgagggtaaaagaactttccgctaagcgatagactgtatgtaaacacagtattgcaaggacgcggaacatgcctcatgtggcggccctcgcgagaattaattcagataaaaaaaatccttagctttcgctaaggatgatttctagcgatgaccctgctgattggttcgctgaccgtagactggttggcttggtttcatcagccatccgcttgccctcatctgttacgccggcggtagccggccagcctcgcagagcaggattcccgttgagcaccgccaggtgcgaataagggacagtgaagaaggaacacccgctcgcgggtgggcctacttcacctatcctgcccggctgacgccgttggatacaccaaggaaagtctacacgaaccctttggcaaaatcctgtatatcgtgcgacatcgcgcgcgcgcgcgcggatgctagtacgttgtgtctcaaaatctctgatgttacattgcacaagataaaaatatatcatcatgaacaataaaactgtctgcttacataaacagtaatacaaggggtgttatgagccatattcaacgggaaacgtcttgctcgaggccgcgattaaattccaacatggatgctgatttatatgggtataaatgggctcgcgataatgtcgggcaatcaggtgcgacaatctatcgattgtatgggaagcccgatgcgccagagttgtttctgaaacatggcaaaggtagcgttgccaatgatgttacagatgagatggtcagactaaactggctgacggaatttatgcctcttccgaccatcaagcattttatccgtactcctgatgatgcatggttactcaccactgcgatccccgggaaaacagcattccaggtattagaagaatatcctgattcaggtgaaaatattgttgatgcgctggcagtgttcctgcgccggttgcattcgattcctgtttgtaattgtccttttaacagcgatcgcgtatttcgtctcgctcaggcgcaatcacgaatgaataacggtttggttgatgcgagtgattttgatgacgagcgtaatggctggcctgttgaacaagtctggaaagaaatgcataagcttttgccattctcaccggattcagtcgtcactcatggtgatttctcacttgataaccttatttttgacgaggggaaattaataggttgtattgatgttggacgagtcggaatcgcagaccgataccaggatcttgccatcctatggaactgcctcggtgagttttctccttcattacagaaacggctttttcaaaaatatggtattgataatcctgatatgaataaattgcagtttcatttgatgctcgatgagtttttctaatcagaattggttaattggttgtaacactggcagagcattacgctgacttgacgggacggcggctttgttgaataaatcgaacttttgctgagttgaaggatcagatcacgcatcttcccgacaacgcagaccgttccgtggcaaagcaaaagttcaaaatcaccaactggtccacctacaacaaagctctcatcaaccgtggctccctcactttctggctggatgatggggcgattcaggcctggtatgagtcagcaacaccttcttcacgaggcagacctcagcgctattctgaccttgccatcacgactgtgctggtcattaaacgcgtattcaggctgaccctgcgcgctgcgcagggctttattgattccatttttacactgatgaatgttccgttgcgctgcccggattacagatcctctagataatgaattctataggtaccataaataaggttttcccctgatgctgccacgcgtgactagtatgtggagccacccgcagttcgaaaaaggatcaagcaaaggagaagaacttttcactggatccaagctttctagaatcgggggcccccggggggattctagaacaatgga

SEQ ID NO: 27 - DNA, 8359 bp, Artificial Sequence
  plasmid pHM64
agtcctcgtctcgccctcgaattagcccgcttaatgagcgggctttttttgaattaattctcgcgagctggcacgacaggtttcccgactggaaagcgggcagtgagcgcaacgcaattaatgtaagttagcgcgaattgcaagctggccgacgcgctgggctacgtcttgctggcgttcgggagcagaagagcatacatctggaagcaaagccaggaaagcggcctatggagctgtgcggcagcgctcagtaggcaatttttcaaaatattgttaagccttttctgagcatggtatttttcatggtattaccaattagcaggaaaataagccattgaatataaaagataaaaatgtcttgtttacaatagagtggggggggtcagcctgccgccttgggccgggtgatgtcgtacttgcccgccgcgaactcggttaccgtccagcccagcgcgaccagctccggcaacgcctcgcgcacccgctggcggcgcttgcgcatggtcgaaccactggcctctgacggccagacatagccgcacaaggtatctatggaagccttgccggttttgccggggtcgatccagccacacagccgctggtgcagcaggcgggcggtttcgctgtccagcgcccgcacctcgtccatgctgatgcgcacatgctggccgccacccatgacggcctgcgcgatcaaggggttcagggccacgtacaggcgcccgtccgcctcgtcgctggcgtactccgacagcagccgaaacccctgccgcttgcggccattctgggcgatgatggataccttccaaaggcgctcgatgcagtcctgtatgtgcttgagcgccccaccactatcgacctctgccccgatttcctttgccagcgcccgatagctacctttgaccaccatggcatcagcggtgacggcctcccacttgggttccaggaacagccggagctgccgtccgccttcggtcttgggttccgggccaagcactaggccattaggcccagccatggccaccagcccttgcaggatgcgcagatcatcagcgcccagcggctccgggccgctgaactcgatccgcttgccgtcgccgtagtcatacgtcacgtccagcttgctgcgcttgcgctcgccccgcttgagggcacggaacaggccgggggccagacagtgcgccgggtcgtgtcggacgtggctgaggctgtgcttgttcttaggcttcaccacggggcacccccttgctcttgcgctgcctctccagcacggcgggcttgagcaccccgccgtcatgccgcctgaaccaccgatcagcgaacggtgcgccatagttggccttgctcacaccgaagcggacgaagaaccggcgctggtcgtcgtccacaccccattcctcggcctcggcgctggtcatgctcgacaggtaggactgccagcggatgttatcgaccagtaccgagctgccccggctggcctgctgctggtcgcctgcgcccatcatggccgcgcccttgctggcatggtgcaggaacacgatagagcacccggtatcggcggcgatggcctccatgcgaccgatgacctgggccatggggccgctggcgttttcttcctcgatgtggaaccggcgcagcgtgtccagcaccatcaggcggcggccctcggcggcgcgcttgaggccgtcgaaccactccggggccatgatgttgggcaggctgccgatcagcggctggatcagcaggccgtcagccacggcttgccgttcctcggcgctgaggtgcgccccaagggcgtgcaggcggtgatgaatggcggtgggcgggtcttcggcgggcaggtagatcaccgggccggtgggcagttcgcccacctccagcagatccggcccgcctgcaatctgtgcggccagttgcagggccagcatggatttaccggcaccaccgggcgacaccagcgccccgaccgtaccggccaccatgttgggcaaaacgtagtccagcggtggcggcgctgctgcgaacgcctccagaatattgataggcttatgggtagccattgattgcctcctttgcaggcagttggtggttaggcgctggcggggtcactacccccgccctgcgccgctctgagttcttccaggcactcgcgcagcgcctcgtattcgtcgtcggtcagccagaacttgcgctgacgcatccctttggccttcatgcgctcggcatatcgcgcttggcgtacagcgtcagggctggccagcaggtcgccggtctgcttgtccttttggtctttcatatcagtcaccgagaaacttgccggggccgaaaggcttgtcttcgcggaacaaggacaaggtgcagccgtcaaggttaaggctggccatatcagcgactgaaaagcggccagcctcggccttgtttgacgtataaccaaagccaccgggcaaccaatagcccttgtcacttttgatcaggtagaccgaccctgaagcgcttttttcgtattccataaaacccccttctgtgcgtgagtactcatagtataacaggcgtgagtaccaacgcaagcactacatgctgaaatctggcccgcccctgtccatgcctcgctggcggggtgccggtgcccgtgccagctcggcccgcgcaagctggacgctgggcagacccatgaccttgctgacggtgcgctcgatgtaatccgcttcgtggccgggcttgcgctctgccagcgctgggctggcctcggccatggccttgccgatttcctcggcactgcggccccggctggccagcttctgcgcggcgataaagtcgcacttgctgaggtcatcaccgaagcgcttgaccagcccggccatctcgctgcggtactcgtccagcgccgtgcgccggtggcggctaagctgccgctcggacagttcgaggctggccagcctgcgggccttctcctgctgccgctgggcctgctcgatctgctggccagcctgctgcaccagcgccgggccagcggtggcggtcttgcccttggattcacgcagcagcacccacggctgataaccggcgcgggtggtgtgcttgtccttgcggttggtgaagcccgccaagcggccatagtggcggctgtcggcgctggccgggtcggcgtcgtactcgctggccagcgtccgggcaatctgcccccgaagttcaccgcctgcggcgtcggccaccttgacccatgcctgatagttcttcgggctggtttccactaccagggcaggctcccggccctcggctttcatgtcatccaggtcaaactcgctgaggtcgtccaccagcaccagaccatgccgctcctgctcggcgggcctgatatacacgtcattgccctgggcattcatccgcttgagccatggcgtgttctggagcacttcggcggctgaccattcccggttcatcatctggccggtggtggcgtccctgacgccgatatcgaagcgctcacagcccatggccttgagctgtcggcctatggcctgcaaagtcctgtcgttcttcatcgggccaccaagcgcagccagatcgagccgtcctcggttgtcagtggcgtcaggtcgagcaagagcaacgatgcgatcagcagcaccaccgtaggcatcatggaagccagcatcacggttagccatagcttccagtgccacccccgcgacgcgctccgggcgctctgcgcggcgctgctcacctcggcggctacctcccgcaactctttggccagctccacccatgccgcccctgtctggcgctgggctttcagccactccgccgcctgcgcctcgctggcctgctgggtctggctcatgacctgccgggcttcgtcggccagtgtcgccatgctctgggccagcggttcgatctgctccgctaactcgttgatgcctctggatttcttcactctgtcgattgcgttcatggtctattgcctcccggtattcctgtaagtcgatgatctgggcgttggcggtgtcgatgttcagggccacgtctgcccggtcggtgcggatgccccggccttccatctccaccacgttcggccccaggtgaacaccgggcaggcgctcgatgccctgcgcctcaagtgttctgtggtcaatgcgggcgtcgtggcctgcccgctctaatgcccggttggcatggtcggcccatgcctcgcgggtctgctcaagccatgccttgggcttgagcgcttcggtcttctgtgccccgcccttctccggggtcttgccgttgtaccgcttgaaccactgagcggcgggccgctcgatgccgtcattgatccgctcggagatcatcaggtggcagtgcgggttctcgccgccaccggcatggatggccagcgtatacggcaggcgctcggcaccggtcaggtgctgggcgaactcggacgccagcgccttctgctggtcgagggtcagctcgaccggcagggcaaattcgacctccttgaacagccgcccattggcgcgttcatacaggtcggcagcatcccagtagtcggcgggccgctcgacgaactccggcatgtgcccggattcggcgtgcaagacttcatccatgtcgcgggcatacttgccttcgcgctggatgaagtcggccttggccctggccgattggccgcccgacctgctgccggttttcgccgtaaggtgataaatcgccatgctgcctcgctgttgcttttgcttttcggctccatgcaatggccctcggagagcgcaccgcccgaagggtggccgttaggccagtttctcgaagagaaaccggtaagtgcgccctcccctacaaagtagggtcgggattgccgccgctgtgcctccatgatagcctacgagacagcacattaacaatggggtgtcaagatggttaaggggagcaacaaggcggcggatcggctggccaagctcgaagaacaacgagcgcgaatcaatgccgaaattcagcgggtgcgggcaagggaacagcagcaagagcgcaagaacgaaacaaggcgcaaggtgctggtgggggccatgattttggccaaggtgaacagcagcgagtggccggaggatcggctcatggcggcaatggatgcgtaccttgaacgcgaccacgaccgcgccttgttcggtctgccgccacgccagaaggatgagccgggctgaatgatcgaccgagacaggccctgcggggctgcacacgcgcccccacccttcgggtagggggaaaggccgctaaagcggctaaaagcgctccagcgtatttctgcggggtttggtgtggggtttagcgggctttgcccgcctttccccctgccgcgcagcggtggggcggtgtgtagcctagcgcagcgaatagaccagctatccggcctctggccgggcatattgggcaagggcagcagcgccccacaagggcgctgataaccgcgcctagtggattattcttagataatcatggatggatttttccaacaccccgccagcccccgcccctgctgggtttgcaggtttgggggcgtgacagttattgcaggggttcgtgacagttattgcaggggggcgtgacagttattgcaggggttcgtgacagttagtacgggagtgacgggcactggctggcaatgtctagcaacggcaggcatttcggctgagggtaaaagaactttccgctaagcgatagactgtatgtaaacacagtattgcaaggacgcggaacatgcctcatgtggcggccctcgcgagaattaattcagataaaaaaaatccttagctttcgctaaggatgatttctagcgatgaccctgctgattggttcgctgaccgtagactggttggcttggtttcatcagccatccgcttgccctcatctgttacgccggcggtagccggccagcctcgcagagcaggattcccgttgagcaccgccaggtgcgaataagggacagtgaagaaggaacacccgctcgcgggtgggcctacttcacctatcctgcccggctgacgccgttggatacaccaaggaaagtctacacgaaccctttggcaaaatcctgtatatcgtgcgacatcgcgcgcgcgcgcgcggatgctagtacgttgtgtctcaaaatctctgatgttacattgcacaagataaaaatatatcatcatgaacaataaaactgtctgcttacataaacagtaatacaaggggtgttatgagccatattcaacgggaaacgtcttgctcgaggccgcgattaaattccaacatggatgctgatttatatgggtataaatgggctcgcgataatgtcgggcaatcaggtgcgacaatctatcgattgtatgggaagcccgatgcgccagagttgtttctgaaacatggcaaaggtagcgttgccaatgatgttacagatgagatggtcagactaaactggctgacggaatttatgcctcttccgaccatcaagcattttatccgtactcctgatgatgcatggttactcaccactgcgatccccgggaaaacagcattccaggtattagaagaatatcctgattcaggtgaaaatattgttgatgcgctggcagtgttcctgcgccggttgcattcgattcctgtttgtaattgtccttttaacagcgatcgcgtatttcgtctcgctcaggcgcaatcacgaatgaataacggtttggttgatgcgagtgattttgatgacgagcgtaatggctggcctgttgaacaagtctggaaagaaatgcataagcttttgccattctcaccggattcagtcgtcactcatggtgatttctcacttgataaccttatttttgacgaggggaaattaataggttgtattgatgttggacgagtcggaatcgcagaccgataccaggatcttgccatcctatggaactgcctcggtgagttttctccttcattacagaaacggctttttcaaaaatatggtattgataatcctgatatgaataaattgcagtttcatttgatgctcgatgagtttttctaatcagaattggttaattggttgtaacactggcagagcattacgctgacttgacgggacggcggctttgttgaataaatcgaacttttgctgagttgaaggatcagatcacgcatcttcccgacaacgcagaccgttccgtggcaaagcaaaagttcaaaatcaccaactggtccacctacaacaaagctctcatcaaccgtggctccctcactttctggctggatgatggggcgattcaggcctggtatgagtcagcaacaccttcttcacgaggcagacctcagcgctattctgaccttgccatcacgactgtgctggtcattaaacgcgtattcaggctgaccctgcgcgctgcgcagggctttattgattccatttttacactgatgaatgttccgttgcgctgcccggattacagatcctctagataatgaattctataggtaccttgacggctagctcagtcctaggtatagtgctagcactagagaaagaggggaaatactagtatgcaccatcaccatcaccatgaaaacctttacttccagagcatggcgactgggtcccgcacttcattgttgctggcatttggacttctttgtctgccttggttgcaggaggggagtgcttttcccactataccattatctcgtctgttcgacaacgcgatgttacgggctcacagacttcaccaattagcttttgatacataccaagagtttgaggaagcctatataccaaaggaacaaaagtattcatttcttcaaaatccgcaaaccagtctttgcttcagcgagagtataccaacaccgtccaaccgtgaggaaacacaacagaagagcaacttagaacttcttcgtatttctcttttgttaatacagtcatggttggaacccgtgcagttcctgagatctgtttttgccaattcactggtctacggtgcatccgatagtaatgtgtacgatttattgaaggacttggaagagggcatccagacgttgatgggtcggcttgaagacggttcgcccagaactggccaaatatttaagcaaacatattccaagttcgacacaaattctcataatgacgatgcactgttgaagaactatggtcttttatactgtttccgcaaggatatggataaagtggaaacatttctgcgtattgtccagtgtcgctcggttgaaggttcctgcggattttagggatcctgaagatccaacgctcggttgccgccgggcgttttttattctgcaggagcagaagagcatacatctggaagctttctagaatcgggggcccccggggggattctagaacaatgga

SEQ ID NO: 28 - DNA, 80 bp, Artificial Sequence
  Primer DNA_174
ataatgaattctataggtaccataaataaggttttcccctgatgctgccacgcgtgactagtatgtggagccacccgcag

SEQ ID NO: 29 - DNA, 39 bp, Artificial Sequence
  Primer DNA_053
tttggtctcaagcttggatccagtgaaaagttcttctcc

SEQ ID NO: 30 - DNA, 71 bp, Artificial Sequence
  Primer Primer DNA_044
tgtccctcccctcttttgttatttaccgtctctagtgctagcattatacctaggactgagctagctgtcaa